European Patent Application EP 4 545 081 A1, published April 30, 2025. Title: Ligand modulating adenosine receptor and composition for preventing, improving or treating obesity comprising thereof. Applicant: Seoul National University R&DB Foundation. Application KR. The sequence listing filed with the application follows.

SEQUENCE LISTING (14 sequences)

SEQ ID NO: 1 - DNA, 19 bp, synthetic construct
  source 1..19: mol_type = other DNA
tggcctctcagtggatgtg

SEQ ID NO: 2 - DNA, 21 bp, synthetic construct
  source 1..21: mol_type = other DNA
cgtggtctcccagcatagaag

SEQ ID NO: 3 - DNA, 21 bp, synthetic construct
  source 1..21: mol_type = other DNA
tgctcttctgtatcgcccagt

SEQ ID NO: 4 - DNA, 21 bp, synthetic construct
  source 1..21: mol_type = other DNA
gccgtgttaaggaatctgctg

SEQ ID NO: 5 - DNA, 20 bp, synthetic construct
  source 1..20: mol_type = other DNA
gtggtctttgggaaggtgaa

SEQ ID NO: 6 - DNA, 20 bp, synthetic construct
  source 1..20: mol_type = other DNA
ttacaggacattgcgagcag

SEQ ID NO: 7 - DNA, 20 bp, synthetic construct
  source 1..20: mol_type = other DNA
tggctcagttcgtgcatcat

SEQ ID NO: 8 - DNA, 20 bp, synthetic construct
  source 1..20: mol_type = other DNA
atccttacccatcgactgcc

SEQ ID NO: 9 - DNA, 21 bp, synthetic construct
  source 1..21: mol_type = other DNA
cagagaagggaagcaatcgca

SEQ ID NO: 10 - DNA, 21 bp, synthetic construct
  source 1..21: mol_type = other DNA
accatgacttctacagggggt

SEQ ID NO: 11 - DNA, 20 bp, synthetic construct
  source 1..20: mol_type = other DNA
gcgtcccgctcaggtataaa

SEQ ID NO: 12 - DNA, 20 bp, synthetic construct
  source 1..20: mol_type = other DNA
caatgccaaaggcaaggacc

SEQ ID NO: 13 - DNA, 20 bp, synthetic construct
  source 1..20: mol_type = other DNA
agtaagaacggtggccctct

SEQ ID NO: 14 - DNA, 21 bp, synthetic construct
  source 1..21: mol_type = other DNA
atccctgccttcccattaacc